European Patent Specification EP 3 441 458 B9, published August 23, 2023. Title: Culture Medium For Epithelial Stem Cells And Organoids Comprising Said Stem Cells. Applicant: Koninklijke Nederlandse Akademie van Wetenschappen. The sequence listing filed with the application follows.

SEQUENCE LISTING (45 sequences)

SEQ ID NO: 1 - protein, 17 aa, H. sapiens
CDDYYYGFGCNKFCRPR

SEQ ID NO: 2 - DNA, 24 bp, Artificial Sequence
  Primer
tattgtatctaccgtgaatcttgg

SEQ ID NO: 3 - DNA, 18 bp, Artificial Sequence
  Primer
cagttgtccgtggctctc

SEQ ID NO: 4 - DNA, 18 bp, Artificial Sequence
  Primer
tccaacctcagcgtcttc

SEQ ID NO: 5 - DNA, 18 bp, Artificial Sequence
  Primer
tgggaatgtgtgtcaaag

SEQ ID NO: 6 - DNA, 20 bp, Artificial Sequence
  Primer
aagtttgttgttggatatgc

SEQ ID NO: 7 - DNA, 21 bp, Artificial Sequence
  Primer
catcttaggctttgtatttgg

SEQ ID NO: 8 - DNA, 20 bp, Artificial Sequence
  Primer
tcctcggagcttttctacga

SEQ ID NO: 9 - DNA, 20 bp, Artificial Sequence
  Primer
tgtgtctctggggacacttg

SEQ ID NO: 10 - DNA, 20 bp, Artificial Sequence
  Primer
aacaacctgcctatgcaacc

SEQ ID NO: 11 - DNA, 20 bp, Artificial Sequence
  Primer
acttggacgggaactgacac

SEQ ID NO: 12 - DNA, 18 bp, Artificial Sequence
  Primer
aagatcattggcggaaag

SEQ ID NO: 13 - DNA, 19 bp, Artificial Sequence
  Primer
gagtgctcaggatgttaag

SEQ ID NO: 14 - DNA, 21 bp, Artificial Sequence
  Primer
gctgacagcagagaagcggct

SEQ ID NO: 15 - DNA, 21 bp, Artificial Sequence
  Primer
gacaggctctctagctcctgg

SEQ ID NO: 16 - DNA, 20 bp, Artificial Sequence
  Primer
aagttggaagaggaagtcag

SEQ ID NO: 17 - DNA, 18 bp, Artificial Sequence
  Primer
agaccttctgctcagtcg

SEQ ID NO: 18 - DNA, 20 bp, Artificial Sequence
  Primer
tttgtcaagcagcacctttg

SEQ ID NO: 19 - DNA, 20 bp, Artificial Sequence
  Primer
tctacaatgccacgcttctg

SEQ ID NO: 20 - DNA, 20 bp, Artificial Sequence
  Primer
gaggcaaggaagatgctgtc

SEQ ID NO: 21 - DNA, 20 bp, Artificial Sequence
  Primer
gggcatcattctctgtctgg

SEQ ID NO: 22 - DNA, 22 bp, Artificial Sequence
  Primer
ttactttgtggctggattgctt

SEQ ID NO: 23 - DNA, 21 bp, Primer
agtggcgtttgtcttcattca

SEQ ID NO: 24 - DNA, 22 bp, Artificial Sequence
  Primer
ggaaatgctttgacacacattc

SEQ ID NO: 25 - DNA, 23 bp, Artificial Sequence
  Primer
ggaagtcatcaaggttattataa

SEQ ID NO: 26 - DNA, 20 bp, Artificial Sequence
  Primer
tgaatcctcggccttctatg

SEQ ID NO: 27 - DNA, 22 bp, Artificial Sequence
  Primer
cagttaaagttggtggcacttc

SEQ ID NO: 28 - DNA, 20 bp, Artificial Sequence
  Primer
ccaacctgtgggtgtcttct

SEQ ID NO: 29 - DNA, 20 bp, Artificial Sequence
  Primer
ttagggacctggatgctttg

SEQ ID NO: 30 - DNA, 20 bp, Artificial Sequence
  Primer
tgcatgctcaatggtatggt

SEQ ID NO: 31 - DNA, 20 bp, Artificial Sequence
  Primer
tgtgggctctggagaagagt

SEQ ID NO: 32 - DNA, 20 bp, Artificial Sequence
  Primer
ccatgaagtgggagtgtgtg

SEQ ID NO: 33 - DNA, 20 bp, Artificial Sequence
  Primer
ttgggatagcatccttccag

SEQ ID NO: 34 - DNA, 22 bp, Artificial Sequence
  Primer
gcccagcagagaaaggaatcca

SEQ ID NO: 35 - DNA, 20 bp, Artificial Sequence
  Primer
gcgcctctttgacctcttcc

SEQ ID NO: 36 - DNA, 20 bp, Artificial Sequence
  Primer
gccaactattccccagctct

SEQ ID NO: 37 - DNA, 20 bp, Artificial Sequence
  Primer
ggctctggaagagtgttgct

SEQ ID NO: 38 - DNA, 20 bp, Artificial Sequence
  Primer
gaggcaaggaagatgctgtc

SEQ ID NO: 39 - DNA, 20 bp, Artificial Sequence
  Primer
gggcatcattctctgtctgg

SEQ ID NO: 40 - DNA, 20 bp, Artificial Sequence
  Primer
gaacggggccatggtcagca

SEQ ID NO: 41 - DNA, 20 bp, Artificial Sequence
  Primer
cataattggtcttgcatgcc

SEQ ID NO: 42 - DNA, 19 bp, Artificial Sequence
  Primer
cttgctgcagacgctcaac

SEQ ID NO: 43 - DNA, 20 bp, Artificial Sequence
  Primer
tctgtgtacaccacccggta

SEQ ID NO: 44 - DNA, 20 bp, Artificial Sequence
  Primer
aagcttgctggtgaaaagga

SEQ ID NO: 45 - DNA, 20 bp, Artificial Sequence
  Primer
ttgcgctcatcttaggcttt